European Patent Application EP 4 506 361 A1, published February 12, 2025. Title: Antibody against c-Met and use thereof. Applicant: BIOTHEUS INC. The sequence listing filed with the application follows.

SEQUENCE LISTING (122 sequences)

SEQ ID NO: 1 - protein, 120 aa, synthetic construct
QVQLVQSGAEVKKPGASVKVSCKTSGYTFTNYGISWVRQAPGQGLEWMGWISAYNGHTNYAQKLQGRVTMTTDTSTSTAYMELRSLRSDDTAVYYCARDRRTGTSFFDYWGQGTLVTVSS

SEQ ID NO: 2 - protein, 107 aa, synthetic construct
DIVMTQSPSSVSASVGDRVTITCRASQGISSWLAWYQQKPGKAPKLLIYAASSLQSGVPSKFSGSGSGTEFTLTISSLQPEDFATYFCQQAYGFPLTFGGGTKVEIK

SEQ ID NO: 3 - protein, 121 aa, synthetic construct
EVQLVESGGGLVQPGGSLRLSCAASGFTFSSYAMTWVRQAPGKGLEWVSVISGSGGTTYYADSVKGRFTISRDNSKNTLYLQMHSLRAEDTAVYYCAKVITFERGRTFDIWGQGTMVTVSS

SEQ ID NO: 4 - protein, 107 aa, synthetic construct
DIVMTQSPSSLSASVGDRVTITCRASQSFSDYLNWYRQKPGKAPKLLLFAASSLQSGVPSRFSGSGSGTDFTLTISSLQPEDFATYYCQQSYSPPYTFGQGTKLEIK

SEQ ID NO: 5 - protein, 118 aa, synthetic construct
QLQLQESGPGLVKPSETLSLTCTVSGGSISSSSYYWGWIRQSPGKGLEWIGSIYYSGNTYYNPSLKSRVTISVDTSKNQFSLKLSSVTAADTAVYYCVRQVYDFWRDWGQGTLVTVSS

SEQ ID NO: 6 - protein, 107 aa, synthetic construct
DIVMTQSPSSVSASVGDRVTITCRASQGINSWLAWYQQKPGKAPNLLIYAASSLQSGVPSRFSGRGSGTDFSLTISSLHPEDFATYYCQQAKGFPLTFGGGTKVEIK

SEQ ID NO: 7 - protein, 124 aa, synthetic construct
QVQLVQSGAEVKKPGASMKVSCKASGNTFISYGINWVRQAPGQGLEWMGWISAYNGNTNYAQKFQGRVTMTTDTSTSSAYMELRNLRSDDTAVYYCATGDTTSSGYYNYYMDVWGKGTTVTVSS

SEQ ID NO: 8 - protein, 108 aa, synthetic construct
EIVLTQSPGTLSLSPGERATLSCRASQSVSSSYLAWYQQKPGQAPRLLIYGAFSRATGIPDRFSGSGSGTDFTLTISRLEPEDFAVYYCQQYGSSPRTFGQGTKVDIK

SEQ ID NO: 9 - protein, 118 aa, synthetic construct
QVQLQESGPGLVKPSETLSLTCTVSGGSVTSVNYYWKWIRQPPGKGLEWIGYISYSGNTNYNPSLKSRVTISVDTSKNQFSLKLSSVTAADTAVYYCVRAPYYYMDVWSKGTTVTVSS

SEQ ID NO: 10 - protein, 107 aa, synthetic construct
DIVMTQSPSSVSASVGDRVTITCRASQGISSWLAWYQQKPGKAPKLLIYAVSSLQSGVPSRFSGSGSGTDFTLTISSLQPEDFATYFCQQANSFPLTFGGGTKVEIK

SEQ ID NO: 11 - protein, 118 aa, synthetic construct
QLQLQESGPGLVKPSETLSLTCTVSGGSISSSSYYWGWIRQSPGKGLEWIGSRYYSGNTYYNPSLKSRVTMSVDTSKNQFSLKLRSVTAADTAVYYCARQVYDYWRDWGQGALVTVSS

SEQ ID NO: 12 - protein, 107 aa, synthetic construct
DIVMTQSPSSVSASVGDRVTITCRASQGISSWLAWYQQKPGKAPNLLIYAASNLPSGVPSRFSGSGSGTVFTLTISSLQPEDFATYYCQQSNSFPLTFGGGTKVEIK

SEQ ID NO: 13 - protein, 121 aa, synthetic construct
EVQLVESGGGLVQPGGSLRLFCGASGFTFSSYAMSWVRQAPGKGLEWVSAITGSGGSTYYADSVKGRFTISRDNSKNTLFLQLNSLRAEDTAIYYCAKIVTVEAGRWLDPWGQGTMVTVSS

SEQ ID NO: 14 - protein, 107 aa, synthetic construct
DIRMTQSPSSLSASVGDRVTITCRASQSISNYLNWFQQKPGKAPKLLIYATSSLQSGVPSRFSGSGSGTDFTLTISSLQPEDFATYYCQQSYSIPYTFGQGTKVEIK

SEQ ID NO: 15 - protein, 121 aa, synthetic construct
EVQLLESGGGLVQPGGSLRLSCAASGFTFSSYAMTWVRQAPGKGLEWVSVISGSGGSTYYEDSVKGRFTISRDNSKNTLYLQMNSLRAEDTAVYYCAKVITFERGRTFDIWGQGTMVTVSS

SEQ ID NO: 16 - protein, 108 aa, synthetic construct
EIVLTQSPGTLSLSPGERATLSCRASQSVSSSYLAWYQQKPGQAPRLLIYGPSSRATGIPDRFSGSGSGTDFTLTISSLQPADFASYYCQQSYITPYTFGQGTKVEIK

SEQ ID NO: 17 - protein, 121 aa, synthetic construct
EVQLVESGGGLVQPGGSLRLSCAASGFTFRNYAMSWVRQAPGKGLEWVSAISGSGVGTYYADSVKGRFTISRDNSKNTLFLQMNSLRVEDTAVYYCVRVMTVEFSRWLDPWGQGTLVTVSS

SEQ ID NO: 18 - protein, 107 aa, synthetic construct
DIQLTQSPSSLSASVGDRVTITCRASQSIITYLNWYQQKPGKAPKLLIYAASSLQSGVPSRFSGSGSGTDFTLNISSLQPEDFATYYCQQANSLPYTFGQGTKVEIK

SEQ ID NO: 19 - protein, 8 aa, synthetic construct
GYTFTNYG

SEQ ID NO: 20 - protein, 6 aa, synthetic construct
QGISSW

SEQ ID NO: 21 - protein, 8 aa, synthetic construct
GFTFSSYA

SEQ ID NO: 22 - protein, 6 aa, synthetic construct
QSFSDY

SEQ ID NO: 23 - protein, 10 aa, synthetic construct
GGSISSSSYY

SEQ ID NO: 24 - protein, 6 aa, synthetic construct
QGINSW

SEQ ID NO: 25 - protein, 8 aa, synthetic construct
GNTFISYG

SEQ ID NO: 26 - protein, 7 aa, synthetic construct
QSVSSSY

SEQ ID NO: 27 - protein, 10 aa, synthetic construct
GGSVTSVNYY

SEQ ID NO: 28 - protein, 6 aa, synthetic construct
QGISSW

SEQ ID NO: 29 - protein, 10 aa, synthetic construct
GGSISSSSYY

SEQ ID NO: 30 - protein, 6 aa, synthetic construct
QGISSW

SEQ ID NO: 31 - protein, 8 aa, synthetic construct
GFTFSSYA

SEQ ID NO: 32 - protein, 6 aa, synthetic construct
QSISNY

SEQ ID NO: 33 - protein, 8 aa, synthetic construct
GFTFSSYA

SEQ ID NO: 34 - protein, 7 aa, synthetic construct
QSVSSSY

SEQ ID NO: 35 - protein, 8 aa, synthetic construct
GFTFRNYA

SEQ ID NO: 36 - protein, 6 aa, synthetic construct
QSIITY

SEQ ID NO: 37 - protein, 8 aa, synthetic construct
ISAYNGHT

SEQ ID NO: 38 - skipped

SEQ ID NO: 39 - protein, 8 aa, synthetic construct
ISGSGGTT

SEQ ID NO: 40 - skipped

SEQ ID NO: 41 - protein, 7 aa, synthetic construct
IYYSGNT

SEQ ID NO: 42 - skipped

SEQ ID NO: 43 - protein, 8 aa, synthetic construct
ISAYNGNT

SEQ ID NO: 44 - skipped

SEQ ID NO: 45 - protein, 7 aa, synthetic construct
ISYSGNT

SEQ ID NO: 46 - skipped

SEQ ID NO: 47 - protein, 7 aa, synthetic construct
RYYSGNT

SEQ ID NO: 48 - skipped

SEQ ID NO: 49 - protein, 8 aa, synthetic construct
ITGSGGST

SEQ ID NO: 50 - skipped

SEQ ID NO: 51 - protein, 8 aa, synthetic construct
ISGSGGST

SEQ ID NO: 52 - skipped

SEQ ID NO: 53 - protein, 8 aa, synthetic construct
ISGSGVGT

SEQ ID NO: 54 - skipped

SEQ ID NO: 55 - protein, 13 aa, synthetic construct
ARDRRTGTSFFDY

SEQ ID NO: 56 - protein, 9 aa, synthetic construct
QQAYGFPLT

SEQ ID NO: 57 - protein, 14 aa, synthetic construct
AKVITFERGRTFDI

SEQ ID NO: 58 - protein, 9 aa, synthetic construct
QQSYSPPYT

SEQ ID NO: 59 - protein, 10 aa, synthetic construct
VRQVYDFWRD

SEQ ID NO: 60 - protein, 9 aa, synthetic construct
QQAKGFPLT

SEQ ID NO: 61 - protein, 17 aa, synthetic construct
ATGDTTSSGYYNYYMDV

SEQ ID NO: 62 - protein, 9 aa, synthetic construct
QQYGSSPRT

SEQ ID NO: 63 - protein, 10 aa, synthetic construct
VRAPYYYMDV

SEQ ID NO: 64 - protein, 9 aa, synthetic construct
QQANSFPLT

SEQ ID NO: 65 - protein, 10 aa, synthetic construct
ARQVYDYWRD

SEQ ID NO: 66 - protein, 9 aa, synthetic construct
QQSNSFPLT

SEQ ID NO: 67 - protein, 14 aa, synthetic construct
AKIVTVEAGRWLDP

SEQ ID NO: 68 - protein, 9 aa, synthetic construct
QQSYSIPYT

SEQ ID NO: 69 - protein, 14 aa, synthetic construct
AKVITFERGRTFDI

SEQ ID NO: 70 - protein, 9 aa, synthetic construct
QQSYITPYT

SEQ ID NO: 71 - protein, 14 aa, synthetic construct
VRVMTVEFSRWLDP

SEQ ID NO: 72 - protein, 9 aa, synthetic construct
QQANSLPYT

SEQ ID NO: 73 - DNA, 24 bp, synthetic construct
  source 1..24: mol_type = other DNA
acaggtgcccactcccaggtgcag

SEQ ID NO: 74 - DNA, 23 bp, synthetic construct
  source 1..23: mol_type = other DNA
aaggtgtccagtgtgargtgcag

SEQ ID NO: 75 - DNA, 27 bp, synthetic construct
  source 1..27: mol_type = other DNA
cccagatgggtcctgtcccaggtgcag

SEQ ID NO: 76 - DNA, 24 bp, synthetic construct
  source 1..24: mol_type = other DNA
caaggagtctgttccgaggtgcag

SEQ ID NO: 77 - DNA, 47 bp, synthetic construct
  source 1..47: mol_type = other DNA
tgagcagcagaacctggagccaagggatagacagatggggctgttgt

SEQ ID NO: 78 - DNA, 47 bp, synthetic construct
  source 1..47: mol_type = other DNA
tgagcagcagaacctggagccagtggatagacagatggggctgttgt

SEQ ID NO: 79 - DNA, 25 bp, synthetic construct
  source 1..25: mol_type = other DNA
atgaggstcccygctcagctgctgg

SEQ ID NO: 80 - DNA, 28 bp, synthetic construct
  source 1..28: mol_type = other DNA
ctcttcctcctgctactctggctcccag

SEQ ID NO: 81 - DNA, 25 bp, synthetic construct
  source 1..25: mol_type = other DNA
atttctctgttgctctggatctctg

SEQ ID NO: 82 - DNA, 47 bp, synthetic construct
  source 1..47: mol_type = other DNA
tgttcagaagatggtgggaagatagatacagttggtgcagcatcagc

SEQ ID NO: 83 - DNA, 53 bp, synthetic construct
  source 1..53: mol_type = other DNA
gagaagctgttgctgaagcttctttggacaagagacaggtgcagctggtgcag

SEQ ID NO: 84 - DNA, 53 bp, synthetic construct
  source 1..53: mol_type = other DNA
gagaagctgttgctgaagcttctttggacaagagagaggtgcagctggtgcag

SEQ ID NO: 85 - DNA, 53 bp, synthetic construct
  source 1..53: mol_type = other DNA
gagaagctgttgctgaagcttctttggacaagagagaggtgcagctggtggag

SEQ ID NO: 86 - DNA, 53 bp, synthetic construct
  source 1..53: mol_type = other DNA
gagaagctgttgctgaagcttctttggacaagagagaggtgcagctgttggag

SEQ ID NO: 87 - DNA, 53 bp, synthetic construct
  source 1..53: mol_type = other DNA
gagaagctgttgctgaagcttctttggacaagagacaggtgcagctgcaggag

SEQ ID NO: 88 - DNA, 55 bp, synthetic construct
  source 1..55: mol_type = other DNA
gagaagctgttgctgaagcttctttggacaagagacaggtgcagctacagcagtg

SEQ ID NO: 89 - DNA, 53 bp, synthetic construct
  source 1..53: mol_type = other DNA
gagaagctgttgctgaagcttctttggacaagagacaggttcagctggtgcag

SEQ ID NO: 90 - DNA, 53 bp, synthetic construct
  source 1..53: mol_type = other DNA
gagaagctgttgctgaagcttctttggacaagagacaggtccagctggtacag

SEQ ID NO: 91 - DNA, 53 bp, synthetic construct
  source 1..53: mol_type = other DNA
gagaagctgttgctgaagcttctttggacaagagacaggtgcagctggtggag

SEQ ID NO: 92 - DNA, 53 bp, synthetic construct
  source 1..53: mol_type = other DNA
gagaagctgttgctgaagcttctttggacaagagagaagtgcagctggtggag

SEQ ID NO: 93 - DNA, 53 bp, synthetic construct
  source 1..53: mol_type = other DNA
gagaagctgttgctgaagcttctttggacaagagacagctgcagctgcaggag

SEQ ID NO: 94 - DNA, 53 bp, synthetic construct
  source 1..53: mol_type = other DNA
gagaagctgttgctgaagcttctttggacaagagacaggtacagctgcagcag

SEQ ID NO: 95 - DNA, 53 bp, synthetic construct
  source 1..53: mol_type = other DNA
gccagggggaagaccgatgggcccttggtgctagctgaggagacggtgaccag

SEQ ID NO: 96 - DNA, 55 bp, synthetic construct
  source 1..55: mol_type = other DNA
gccagggggaagaccgatgggcccttggtgctagctgaagagacggtgaccattg

SEQ ID NO: 97 - DNA, 54 bp, synthetic construct
  source 1..54: mol_type = other DNA
gccagggggaagaccgatgggcccttggtgctagctgaggagacggtgaccgtg

SEQ ID NO: 98 - DNA, 51 bp, synthetic construct
  source 1..51: mol_type = other DNA
ccttctttttctctttagctcggcttattccgacatccagatgacccagtc

SEQ ID NO: 99 - DNA, 52 bp, synthetic construct
  source 1..52: mol_type = other DNA
ccttctttttctctttagctcggcttattccgacatccagttgacccagtct

SEQ ID NO: 100 - DNA, 51 bp, synthetic construct
  source 1..51: mol_type = other DNA
ccttctttttctctttagctcggcttattccgatatccggatgacccagtc

SEQ ID NO: 101 - DNA, 51 bp, synthetic construct
  source 1..51: mol_type = other DNA
ccttctttttctctttagctcggcttattccgatattgtgatgacccagac

SEQ ID NO: 102 - DNA, 51 bp, synthetic construct
  source 1..51: mol_type = other DNA
ccttctttttctctttagctcggcttattccgatattgtgatgactcagtc

SEQ ID NO: 103 - DNA, 51 bp, synthetic construct
  source 1..51: mol_type = other DNA
ccttctttttctctttagctcggcttattccgatgttgtgatgactcagtc

SEQ ID NO: 104 - DNA, 51 bp, synthetic construct
  source 1..51: mol_type = other DNA
ccttctttttctctttagctcggcttattccgaaattgtgttgacacagtc

SEQ ID NO: 105 - DNA, 51 bp, synthetic construct
  source 1..51: mol_type = other DNA
ccttctttttctctttagctcggcttattccgaaatagtgatgacgcagtc

SEQ ID NO: 106 - DNA, 52 bp, synthetic construct
  source 1..52: mol_type = other DNA
ccttctttttctctttagctcggcttattccgaaattgtgttgacgcagtct

SEQ ID NO: 107 - DNA, 51 bp, synthetic construct
  source 1..51: mol_type = other DNA
ccttctttttctctttagctcggcttattccgacatcgtgatgacccagtc

SEQ ID NO: 108 - DNA, 53 bp, synthetic construct
  source 1..53: mol_type = other DNA
ggaagatgaagacagatggtgcagccaccgtacgtttgatytccaccttggtc

SEQ ID NO: 109 - DNA, 53 bp, synthetic construct
  source 1..53: mol_type = other DNA
ggaagatgaagacagatggtgcagccaccgtacgtttgatctccagcttggtc

SEQ ID NO: 110 - DNA, 53 bp, synthetic construct
  source 1..53: mol_type = other DNA
ggaagatgaagacagatggtgcagccaccgtacgtttgatatccactttggtc

SEQ ID NO: 111 - protein, 226 aa, synthetic construct
DKTHTCPPCPAPEAAGGPSVFLFPPKPKDTLMISRTPEVTCVVVDVSHEDPEVKFNWYVDGVEVHNAKTKPREEQYNSTYRVVSVLTVLHQDWLNGKEYKCKVSNKALPAPIEKTISKAKGQPREPQVYTLPPCRDELTKNQVSLWCLVKGFYPSDIAVEWESNGQPENNYKTTPPVLDSDGSFFLYSKLTVDKSRWQQGNVFSCSVMHEALHNHYTQKSLSLSPG

SEQ ID NO: 112 - protein, 226 aa, synthetic construct
DKTHTCPPCPAPEAAGGPSVFLFPPKPKDTLMISRTPEVTCVVVDVSHEDPEVKFNWYVDGVEVHNAKTKPREEQYNSTYRVVSVLTVLHQDWLNGKEYKCKVSNKALPAPIEKTISKAKGQPREPQVCTLPPSRDELTKNQVSLSCAVKGFYPSDIAVEWESNGQPENNYKTTPPVLDSDGSFFLVSKLTVDKSRWQQGNVFSCSVMHEALHNHYTQKSLSLSPG

SEQ ID NO: 113 - protein, 448 aa, synthetic construct
QVQLVQSGAEVKKPGASVKVSCETSGYTFTSYGISWVRQAPGHGLEWMGWISAYNGYTNYAQKLQGRVTMTTDTSTSTAYMELRSLRSDDTAVYYCARDLRGTNYFDYWGQGTLVTVSSASTKGPSVFPLAPSSKSTSGGTAALGCLVKDYFPEPVTVSWNSGALTSGVHTFPAVLQSSGLYSLSSVVTVPSSSLGTQTYICNVNHKPSNTKVDKKVEPKSCDKTHTCPPCPAPELLGGPSVFLFPPKPKDTLMISRTPEVTCVVVDVSHEDPEVKFNWYVDGVEVHNAKTKPREEQYNSTYRVVSVLTVLHQDWLNGKEYKCKVSNKALPAPIEKTISKAKGQPREPQVYTLPPCRDELTKNQVSLWCLVKGFYPSDIAVEWESNGQPENNYKTTPPVLDSDGSFFLYSKLTVDKSRWQQGNVFSCSVMHEALHNHYTQKSLSLSPG

SEQ ID NO: 114 - protein, 214 aa, synthetic construct
DIQMTQSPSSVSASVGDRVTITCRASQGISNWLAWFQHKPGKAPKLLIYAASSLLSGVPSRFSGSGSGTDFTLTISSLQPEDFATYYCQQANSFPITFGQGTRLEIKRTVAAPSVFIFPPSDEQLKSGTASVVCLLNNFYPREAKVQWKVDNALQSGNSQESVTEQDSKDSTYSLSSTLTLSKADYEKHKVYACEVTHQGLSSPVTKSFNRGEC

SEQ ID NO: 115 - protein, 226 aa, synthetic construct; identical to SEQ ID NO: 112

SEQ ID NO: 116 - protein, 444 aa, synthetic construct
QVQLVQSGAEVKKPGASVKVSCKASGYTFTDYYMHWVRQAPGQGLEWMGRVNPNRRGTTYNQKFEGRVTMTTDTSTSTAYMELRSLRSDDTAVYYCARANWLDYWGQGTTVTVSSASTKGPSVFPLAPSSKSTSGGTAALGCLVKDYFPEPVTVSWNSGALTSGVHTFPAVLQSSGLYSLSSVVTVPSSSLGTQTYICNVNHKPSNTKVDKKVEPKSCDKTHTCPPCPAPELLGGPSVFLFPPKPKDTLMISRTPEVTCVVVDVSHEDPEVKFNWYVDGVEVHNAKTKPREEQYNSTYRVVSVLTVLHQDWLNGKEYKCKVSNKALPAPIEKTISKAKGQPREPQVYTLPPCRDELTKNQVSLWCLVKGFYPSDIAVEWESNGQPENNYKTTPPVLDSDGSFFLYSKLTVDKSRWQQGNVFSCSVMHEALHNHYTQKSLSLSPG

SEQ ID NO: 117 - protein, 215 aa, synthetic construct
DIQMTQSPSSLSASVGDRVTITCSVSSSVSSIYLHWYQQKPGKAPKLLIYSTSNLASGVPSRFSGSGSGTDFTLTISSLQPEDFATYYCQVYSGYPLTFGGGTKVEIKRTVAAPSVFIFPPSDEQLKSGTASVVCLLNNFYPREAKVQWKVDNALQSGNSQESVTEQDSKDSTYSLSSTLTLSKADYEKHKVYACEVTHQGLSSPVTKSFNRGEC

SEQ ID NO: 118 - protein, 226 aa, synthetic construct; identical to SEQ ID NO: 112

SEQ ID NO: 119 - protein, 448 aa, synthetic construct
EVQLVESGGGLVQPGGSLRLSCAASGYTFTSYWLHWVRQAPGKGLEWVGMIDPSNSDTRFNPNFKDRFTISADTSKNTAYLQMNSLRAEDTAVYYCATYRSYVTPLDYWGQGTLVTVSSASTKGPSVFPLAPSSKSTSGGTAALGCLVKDYFPEPVTVSWNSGALTSGVHTFPAVLQSSGLYSLSSVVTVPSSSLGTQTYICNVNHKPSNTKVDKKVEPKSCDKTHTCPPCPAPELLGGPSVFLFPPKPKDTLMISRTPEVTCVVVDVSHEDPEVKFNWYVDGVEVHNAKTKPREEQYNSTYRVVSVLTVLHQDWLNGKEYKCKVSNKALPAPIEKTISKAKGQPREPQVYTLPPCRDELTKNQVSLWCLVKGFYPSDIAVEWESNGQPENNYKTTPPVLDSDGSFFLYSKLTVDKSRWQQGNVFSCSVMHEALHNHYTQKSLSLSPG

SEQ ID NO: 120 - protein, 220 aa, synthetic construct
DIQMTQSPSSLSASVGDRVTITCKSSQSLLYTSSQKNYLAWYQQKPGKAPKLLIYWASTRESGVPSRFSGSGSGTDFTLTISSLQPEDFATYYCQQYYAYPWTFGQGTKVEIKRTVAAPSVFIFPPSDEQLKSGTASVVCLLNNFYPREAKVQWKVDNALQSGNSQESVTEQDSKDSTYSLSSTLTLSKADYEKHKVYACEVTHQGLSSPVTKSFNRGEC

SEQ ID NO: 121 - protein, 103 aa, synthetic construct
ASTKGPSVFPLAPSSKSTSGGTAALGCLVKDYFPEPVTVSWNSGALTSGVHTFPAVLQSSGLYSLSSVVTVPSSSLGTQTYICNVNHKPSNTKVDKKVEPKSC

SEQ ID NO: 122 - protein, 107 aa, synthetic construct [sequence omitted]